European Patent Application EP 4 559 999 A1, published May 28, 2025. Title: WASCH- UND REINIGUNGSMITTEL ENTHALTEND ANTIMIKROBIELLES PEPTID. Applicant: Henkel AG & Co. KGaA. Application EP. The sequence listing filed with the application follows.

SEQUENCE LISTING (5 sequences)

SEQ ID NO: 1 - protein, 12 aa, synthetic construct
ILRWPWWPWRRK

SEQ ID NO: 2 - protein, 25 aa, synthetic construct
FSTKTRNWFSEHFKKVKEKLKDTFA

SEQ ID NO: 3 - protein, 22 aa, synthetic construct
KTRNWFSEHFKKVKEKLKDTFA

SEQ ID NO: 4 - protein, 17 aa, synthetic construct
WRWAKWGLKLLKYKKIY

SEQ ID NO: 5 - protein, 17 aa, synthetic construct
IWWAKWGLKLLRYRRWY